European Patent Application EP 4 596 581 A1, published August 6, 2025. Title: ANTI-CD16A ANTIBODY AND APPLICATION THEREOF. Applicant: HEFEI TG IMMUNOPHARMA CO., LTD. Application EP 23881112.9, filed April 4, 2023. The sequence listing filed with the application follows.

SEQUENCE LISTING (62 sequences)

SEQ ID NO: 1 - protein, 6 aa, synthetic construct
SDYAWN

SEQ ID NO: 2 - protein, 16 aa, synthetic construct
YISYSGYTNYNPSLES

SEQ ID NO: 3 - protein, 11 aa, synthetic construct
EVGLRLGWFAY

SEQ ID NO: 4 - protein, 11 aa, synthetic construct
KASQSVNNDVA

SEQ ID NO: 5 - protein, 7 aa, synthetic construct
YASNRYT

SEQ ID NO: 6 - protein, 9 aa, synthetic construct
QQHYSSPWT

SEQ ID NO: 7 - protein, 30 aa, synthetic construct
DVQLQESGPGLVKPSQSLSLTCTVTGYSIT

SEQ ID NO: 8 - protein, 14 aa, synthetic construct
WIRQFPGNKLEWMG

SEQ ID NO: 9 - protein, 32 aa, synthetic construct
RISVTRDTSKNQFFLQLNSVTTEDTATYYCAR

SEQ ID NO: 10 - protein, 11 aa, synthetic construct
WGQGTLVAVSA

SEQ ID NO: 11 - protein, 23 aa, synthetic construct
SIVMTQTPKFLLISAGDRVTITC

SEQ ID NO: 12 - protein, 15 aa, synthetic construct
WYQQKPGQSPKLLIY

SEQ ID NO: 13 - protein, 32 aa, synthetic construct
GVPDHFTGSGYGTDFTFTISTVQAEDLAVYFC

SEQ ID NO: 14 - protein, 10 aa, synthetic construct
FGGGTKLEFK

SEQ ID NO: 15 - protein, 30 aa, synthetic construct
QVQLQESGPGLVKPSETLSLTCTVSGYSIT

SEQ ID NO: 16 - protein, 14 aa, synthetic construct
WIRQPPGKGLEWMG

SEQ ID NO: 17 - protein, 32 aa, synthetic construct
RVTISRDTSKNQFSLKLSSVTAADTAVYYCAR

SEQ ID NO: 18 - protein, 11 aa, synthetic construct
WGQGTLVTVSS

SEQ ID NO: 19 - protein, 23 aa, synthetic construct
DIQMTQSPSSLSASVGDRVTITC

SEQ ID NO: 20 - protein, 15 aa, synthetic construct
WYQQKPGKAPKLLIY

SEQ ID NO: 21 - protein, 32 aa, synthetic construct
GVPSRFSGSGSGTDFTFTISSLQPEDIATYYC

SEQ ID NO: 22 - protein, 10 aa, synthetic construct
FGGGTKLEIK

SEQ ID NO: 23 - protein, 120 aa, synthetic construct
DVQLQESGPGLVKPSQSLSLTCTVTGYSITSDYAWNWIRQFPGNKLEWMGYISYSGYTNYNPSLESRISVTRDTSKNQFFLQLNSVTTEDTATYYCAREVGLRLGWFAYWGQGTLVAVSA

SEQ ID NO: 24 - protein, 107 aa, synthetic construct
SIVMTQTPKFLLISAGDRVTITCKASQSVNNDVAWYQQKPGQSPKLLIYYASNRYTGVPDHFTGSGYGTDFTFTISTVQAEDLAVYFCQQHYSSPWTFGGGTKLEFK

SEQ ID NO: 25 - protein, 120 aa, synthetic construct
QVQLQESGPGLVKPSETLSLTCTVSGYSITSDYAWNWIRQPPGKGLEWMGYISYSGYTNYNPSLESRVTISRDTSKNQFSLKLSSVTAADTAVYYCAREVGLRLGWFAYWGQGTLVTVSS

SEQ ID NO: 26 - protein, 107 aa, synthetic construct
DIQMTQSPSSLSASVGDRVTITCKASQSVNNDVAWYQQKPGKAPKLLIYYASNRYTGVPSRFSGSGSGTDFTFTISSLQPEDIATYYCQQHYSSPWTFGGGTKLEIK

SEQ ID NO: 27 - protein, 330 aa, synthetic construct
AKTTAPSVYPLAPVCGDTTGSSVTLGCLVKGYFPEPVTLTWNSGSLSSGVHTFPAVLQSDLYTLSSSVTVTSSTWPSQSITCNVAHPASSTKVDKKIEPRGPTIKPCPPCKCPAPNLLGGPSVFIFPPKIKDVLMISLSPIVTCVVVDVSEDDPDVQISWFVNNVEVHTAQTQTHREDYNSTLRVVSALPIQHQDWMSGKEFKCKVNNKDLPAPIERTISKPKGSVRAPQVYVLPPPEEEMTKKQVTLTCMVTDFMPEDIYVEWTNNGKTELNYKNTEPVLDSDGSYFMYSKLRVEKKNWVERNSYSCSVVHEGLHNHHTTKSFSRTPGK

SEQ ID NO: 28 - protein, 107 aa, synthetic construct
RADAAPTVSIFPPSSEQLTSGGASVVCFLNNFYPKDINVKWKIDGSERQNGVLNSWTDQDSKDSTYSMSSTLTLTKDEYERHNSYTCEATHKTSTSPIVKSFNRNEC

SEQ ID NO: 29 - protein, 330 aa, synthetic construct [sequence omitted]

SEQ ID NO: 30 - protein, 107 aa, synthetic construct [sequence omitted]

SEQ ID NO: 31 - protein, 450 aa, synthetic construct
DVQLQESGPGLVKPSQSLSLTCTVTGYSITSDYAWNWIRQFPGNKLEWMGYISYSGYTNYNPSLESRISVTRDTSKNQFFLQLNSVTTEDTATYYCAREVGLRLGWFAYWGQGTLVAVSAAKTTAPSVYPLAPVCGDTTGSSVTLGCLVKGYFPEPVTLTWNSGSLSSGVHTFPAVLQSDLYTLSSSVTVTSSTWPSQSITCNVAHPASSTKVDKKIEPRGPTIKPCPPCKCPAPNLLGGPSVFIFPPKIKDVLMISLSPIVTCVVVDVSEDDPDVQISWFVNNVEVHTAQTQTHREDYNSTLRVVSALPIQHQDWMSGKEFKCKVNNKDLPAPIERTISKPKGSVRAPQVYVLPPPEEEMTKKQVTLTCMVTDFMPEDIYVEWTNNGKTELNYKNTEPVLDSDGSYFMYSKLRVEKKNWVERNSYSCSVVHEGLHNHHTTKSFSRTPGK

SEQ ID NO: 32 - protein, 214 aa, synthetic construct
SIVMTQTPKFLLISAGDRVTITCKASQSVNNDVAWYQQKPGQSPKLLIYYASNRYTGVPDHFTGSGYGTDFTFTISTVQAEDLAVYFCQQHYSSPWTFGGGTKLEFKRADAAPTVSIFPPSSEQLTSGGASVVCFLNNFYPKDINVKWKIDGSERQNGVLNSWTDQDSKDSTYSMSSTLTLTKDEYERHNSYTCEATHKTSTSPIVKSFNRNEC

SEQ ID NO: 33 - protein, 450 aa, synthetic construct
DVQLQESGPGLVKPSQSLSLTCTVTGYSITSDYAWNWIRQFPGNKLEWMGYISYSGYTNYNPSLESRISVTRDTSKNQFFLQLNSVTTEDTATYYCAREVGLRLGWFAYWGQGTLVAVSAASTKGPSVFPLAPSSKSTSGGTAALGCLVKDYFPEPVTVSWNSGALTSGVHTFPAVLQSSGLYSLSSVVTVPSSSLGTQTYICNVNHKPSNTKVDKKVEPKSCDKTHTCPPCPAPELLGGPSVFLFPPKPKDTLMISRTPEVTCVVVDVSHEDPEVKFNWYVDGVEVHNAKTKPREEQYNSTYRVVSVLTVLHQDWLNGKEYKCKVSNKALPAPIEKTISKAKGQPREPQVYTLPPSRDELTKNQVSLTCLVKGFYPSDIAVEWESNGQPENNYKTTPPVLDSDGSFFLYSKLTVDKSRWQQGNVFSCSVMHEALHNHYTQKSLSLSPGK

SEQ ID NO: 34 - protein, 214 aa, synthetic construct
SIVMTQTPKFLLISAGDRVTITCKASQSVNNDVAWYQQKPGQSPKLLIYYASNRYTGVPDHFTGSGYGTDFTFTISTVQAEDLAVYFCQQHYSSPWTFGGGTKLEFKRTVAAPSVFIFPPSDEQLKSGTASVVCLLNNFYPREAKVQWKVDNALQSGNSQESVTEQDSKDSTYSLSSTLTLSKADYEKHKVYACEVTHQGLSSPVTKSFNRGEC

SEQ ID NO: 35 - protein, 450 aa, synthetic construct
QVQLQESGPGLVKPSETLSLTCTVSGYSITSDYAWNWIRQPPGKGLEWMGYISYSGYTNYNPSLESRVTISRDTSKNQFSLKLSSVTAADTAVYYCAREVGLRLGWFAYWGQGTLVTVSSASTKGPSVFPLAPSSKSTSGGTAALGCLVKDYFPEPVTVSWNSGALTSGVHTFPAVLQSSGLYSLSSVVTVPSSSLGTQTYICNVNHKPSNTKVDKKVEPKSCDKTHTCPPCPAPELLGGPSVFLFPPKPKDTLMISRTPEVTCVVVDVSHEDPEVKFNWYVDGVEVHNAKTKPREEQYNSTYRVVSVLTVLHQDWLNGKEYKCKVSNKALPAPIEKTISKAKGQPREPQVYTLPPSRDELTKNQVSLTCLVKGFYPSDIAVEWESNGQPENNYKTTPPVLDSDGSFFLYSKLTVDKSRWQQGNVFSCSVMHEALHNHYTQKSLSLSPGK

SEQ ID NO: 36 - protein, 214 aa, synthetic construct
DIQMTQSPSSLSASVGDRVTITCKASQSVNNDVAWYQQKPGKAPKLLIYYASNRYTGVPSRFSGSGSGTDFTFTISSLQPEDIATYYCQQHYSSPWTFGGGTKLEIKRTVAAPSVFIFPPSDEQLKSGTASVVCLLNNFYPREAKVQWKVDNALQSGNSQESVTEQDSKDSTYSLSSTLTLSKADYEKHKVYACEVTHQGLSSPVTKSFNRGEC

SEQ ID NO: 37 - protein, 290 aa, synthetic construct
MGGGAGERLFTSSCLVGLVPLGLRISLVTCPLQCGIMWQLLLPTALLLLVSAGMRTEDLPKAVVFLEPQWYRVLEKDSVTLKCQGAYSPEDNSTQWFHNESLISSQASSYFIDAATVDDSGEYRCQTNLSTLSDPVQLEVHIGWLLLQAPRWVFKEEDPIHLRCHSWKNTALHKVTYLQNGKGRKYFHHNSDFYIPKATLKDSGSYFCRGLFGSKNVSSETVNITITQGLAVSTISSFFPPGYQVSFCLVMVLLFAVDTGLYFSVKTNIRSSTRDWKDHKFKWRKDPQDK

SEQ ID NO: 38 - protein, 254 aa, synthetic construct
MWQLLLPTALLLLVSAGMRAEDLPKAVVFLEPQWYRVLEKDRVTLKCQGAYSPEDNSTRWFHNESLISSQTSSYFIAAARVNNSGEYRCQTSLSTLSDPVQLEVHIGWLLLQAPRWVFKEEESIHLRCHSWKNTLLHKVTYLQNGKGRKYFHQNSDFYIPKATLKDSGSYFCRGLIGSKNVSSETVNITITQDLAVSSISSFFPPGYQVSFCLVMVLLFAVDTGLYFSMKKSIPSSTRDWEDHKFKWSKDPQDK

SEQ ID NO: 39 - DNA, 1350 bp, synthetic construct
  source 1..1350: mol_type = other DNA
caggtgcagctgcaggagtccggccccggcctggtgaagccctccgagaccctgtccctgacctgcaccgtgtccggctactccatcacctccgactacgcctggaactggatcaggcagccccccggcaagggcctggagtggatgggctacatctcctactccggctacaccaactacaacccctccctggagtccagggtgaccatctccagggacacctccaagaaccagttctccctgaagctgtcctccgtgaccgccgccgacaccgccgtgtactactgcgccagggaggtgggcctgaggctgggctggttcgcctactggggccagggcaccctggtgaccgtgtcctccgcctccaccaagggcccctccgtgttccccctggccccctcctccaagtccacctccggcggcaccgccgccctgggctgcctggtgaaggactacttccccgagcccgtgaccgtgtcctggaactccggcgccctgacctccggcgtgcacaccttccccgccgtgctgcagtcctccggcctgtactccctgtcctccgtggtgaccgtgccctcctcctccctgggcacccagacctacatctgcaacgtgaaccacaagccctccaacaccaaggtggacaagaaggtggagcccaagtcctgcgacaagacccacacctgccccccctgccccgcccccgagctgctgggcggcccctccgtgttcctgttcccccccaagcccaaggacaccctgatgatctccaggacccccgaggtgacctgcgtggtggtggacgtgtcccacgaggaccccgaggtgaagttcaactggtacgtggacggcgtggaggtgcacaacgccaagaccaagcccagggaggagcagtacaactccacctacagggtggtgtccgtgctgaccgtgctgcaccaggactggctgaacggcaaggagtacaagtgcaaggtgtccaacaaggccctgcccgcccccatcgagaagaccatctccaaggccaagggccagcccagggagccccaggtgtacaccctgcccccctccagggacgagctgaccaagaaccaggtgtccctgacctgcctggtgaagggcttctacccctccgacatcgccgtggagtgggagtccaacggccagcccgagaacaactacaagaccaccccccccgtgctggactccgacggctccttcttcctgtactccaagctgaccgtggacaagtccaggtggcagcagggcaacgtgttctcctgctccgtgatgcacgaggccctgcacaaccactacacccagaagtccctgtccctgtcccccggcaag

SEQ ID NO: 40 - DNA, 642 bp, synthetic construct
  source 1..642: mol_type = other DNA
gacatccagatgacccagtccccctcctccctgtccgcctccgtgggcgacagggtgaccatcacctgcaaggcctcccagtccgtgaacaacgacgtggcctggtaccagcagaagcccggcaaggcccccaagctgctgatctactacgcctccaacaggtacaccggcgtgccctccaggttctccggctccggctccggcaccgacttcaccttcaccatctcctccctgcagcccgaggacatcgccacctactactgccagcagcactactcctccccctggaccttcggcggcggcaccaagctggagatcaagaggaccgtggccgccccctccgtgttcatcttccccccctccgacgagcagctgaagtccggcaccgcctccgtggtgtgcctgctgaacaacttctaccccagggaggccaaggtgcagtggaaggtggacaacgccctgcagtccggcaactcccaggagtccgtgaccgagcaggactccaaggactccacctactccctgtcctccaccctgaccctgtccaaggccgactacgagaagcacaaggtgtacgcctgcgaggtgacccaccagggcctgtcctcccccgtgaccaagtccttcaacaggggcgagtgc

SEQ ID NO: 41 - protein, 247 aa, synthetic construct
DIQMTQSPSSLSASVGDRVTITCKASQSVNNDVAWYQQKPGKAPKLLIYYASNRYTGVPSRFSGSGSGTDFTFTISSLQPEDIATYYCQQHYSSPWTFGCGTKLEIKGGGGSGGGGSGGGGSGGGGSQVQLQESGPGLVKPSETLSLTCTVSGYSITSDYAWNWIRQPPGKCLEWMGYISYSGYTNYNPSLESRVTISRDTSKNQFSLKLSSVTAADTAVYYCAREVGLRLGWFAYWGQGTLVTVSS

SEQ ID NO: 42 - protein, 244 aa, synthetic construct
DIQMTQSPSSLSASVGDRVTITCSASQDISNYLNWYQQKPGKAPKLLIYYTSNLHSGVPSRFSGSGSGTDFTLTISSLQPEDFATYYCQQYRKLPWTFGQGTKLEIKRGGGGSGGGGSGGGGSQVQLVQSGAEVKKPGSSVKVSCKASGGTFSNYWMHWVRQAPGQGLEWMGATYRGHSDTYYNQKFKGRVTITADKSTSTAYMELSSLRSEDTAVYYCARGAIYDGYDVLDNWGQGTLVTVSS

SEQ ID NO: 43 - protein, 246 aa, synthetic construct
DIVLTQTPLSLSVTPGQPASISCKASQSVDYDGDSYMNWYLQKPGQPPQLLIYAASTLHSGIPDRFSGSGSGTDFTLKISRVEAEDVGVYYCQQSKEDPRTFGQGTKLEIKGGGGSGGGGSGGGGSEVQLVQSGAEVKKPGASVKVSCKASGYTFTDYNMDWVRQAPGQGLEWIGDINPNNGGTLYNQKFRGRVTLTVDTSISTAYMELSRLRSDDTAVYYCARSEVFYGNYADYWGQGTTVTVSS

SEQ ID NO: 44 - protein, 20 aa, synthetic construct
GGGGSGGGGSGGGGSGGGGS

SEQ ID NO: 45 - protein, 232 aa, synthetic construct
EPKSCDKTHTCPPCPAPEAAGGPSVFLFPPKPKDTLMISRTPEVTCVVVDVSHEDPEVKFNWYVDGVEVHNAKTKPREEQYNSTYRVVSVLTVLHQDWLNGKEYKCKVSNKALPAPIEKTISKAKGQPREPQVYTLPPCREEMTKNQVSLWCLVKGFYPSDIAVEWESNGQPENNYKTTPPVLDSDGSFFLYSKLTVDKSRWQQGNVFSCSVMHEALHNHYTQKSLSLSPGK

SEQ ID NO: 46 - protein, 232 aa, synthetic construct
EPKSCDKTHTCPPCPAPEAAGGPSVFLFPPKPKDTLMISRTPEVTCVVVDVSHEDPEVKFNWYVDGVEVHNAKTKPREEQYNSTYRVVSVLTVLHQDWLNGKEYKCKVSNKALPAPIEKTISKAKGQPREPQVCTLPPSREEMTKNQVSLSCAVKGFYPSDIAVEWESNGQPENNYKTTPPVLDSDGSFFLVSKLTVDKSRWQQGNVFSCSVMHEALHNHYTQKSLSLSPGK

SEQ ID NO: 47 - protein, 479 aa, synthetic construct
DIQMTQSPSSLSASVGDRVTITCKASQSVNNDVAWYQQKPGKAPKLLIYYASNRYTGVPSRFSGSGSGTDFTFTISSLQPEDIATYYCQQHYSSPWTFGCGTKLEIKGGGGSGGGGSGGGGSGGGGSQVQLQESGPGLVKPSETLSLTCTVSGYSITSDYAWNWIRQPPGKCLEWMGYISYSGYTNYNPSLESRVTISRDTSKNQFSLKLSSVTAADTAVYYCAREVGLRLGWFAYWGQGTLVTVSSEPKSCDKTHTCPPCPAPEAAGGPSVFLFPPKPKDTLMISRTPEVTCVVVDVSHEDPEVKFNWYVDGVEVHNAKTKPREEQYNSTYRVVSVLTVLHQDWLNGKEYKCKVSNKALPAPIEKTISKAKGQPREPQVYTLPPCREEMTKNQVSLWCLVKGFYPSDIAVEWESNGQPENNYKTTPPVLDSDGSFFLYSKLTVDKSRWQQGNVFSCSVMHEALHNHYTQKSLSLSPGK

SEQ ID NO: 48 - protein, 476 aa, synthetic construct
DIQMTQSPSSLSASVGDRVTITCSASQDISNYLNWYQQKPGKAPKLLIYYTSNLHSGVPSRFSGSGSGTDFTLTISSLQPEDFATYYCQQYRKLPWTFGQGTKLEIKRGGGGSGGGGSGGGGSQVQLVQSGAEVKKPGSSVKVSCKASGGTFSNYWMHWVRQAPGQGLEWMGATYRGHSDTYYNQKFKGRVTITADKSTSTAYMELSSLRSEDTAVYYCARGAIYDGYDVLDNWGQGTLVTVSSEPKSCDKTHTCPPCPAPEAAGGPSVFLFPPKPKDTLMISRTPEVTCVVVDVSHEDPEVKFNWYVDGVEVHNAKTKPREEQYNSTYRVVSVLTVLHQDWLNGKEYKCKVSNKALPAPIEKTISKAKGQPREPQVCTLPPSREEMTKNQVSLSCAVKGFYPSDIAVEWESNGQPENNYKTTPPVLDSDGSFFLVSKLTVDKSRWQQGNVFSCSVMHEALHNHYTQKSLSLSPGK

SEQ ID NO: 49 - protein, 478 aa, synthetic construct
DIVLTQTPLSLSVTPGQPASISCKASQSVDYDGDSYMNWYLQKPGQPPQLLIYAASTLHSGIPDRFSGSGSGTDFTLKISRVEAEDVGVYYCQQSKEDPRTFGQGTKLEIKGGGGSGGGGSGGGGSEVQLVQSGAEVKKPGASVKVSCKASGYTFTDYNMDWVRQAPGQGLEWIGDINPNNGGTLYNQKFRGRVTLTVDTSISTAYMELSRLRSDDTAVYYCARSEVFYGNYADYWGQGTTVTVSSEPKSCDKTHTCPPCPAPEAAGGPSVFLFPPKPKDTLMISRTPEVTCVVVDVSHEDPEVKFNWYVDGVEVHNAKTKPREEQYNSTYRVVSVLTVLHQDWLNGKEYKCKVSNKALPAPIEKTISKAKGQPREPQVCTLPPSREEMTKNQVSLSCAVKGFYPSDIAVEWESNGQPENNYKTTPPVLDSDGSFFLVSKLTVDKSRWQQGNVFSCSVMHEALHNHYTQKSLSLSPGK

SEQ ID NO: 50 - DNA, 1350 bp, synthetic construct
  source 1..1350: mol_type = other DNA
gacgtgcagctgcaggagtccggccccggcctggtgaagccctcccagtccctgtccctgacctgcaccgtgaccggctactccatcacctccgactacgcctggaactggatcaggcagttccccggcaacaagctggagtggatgggctacatctcctactccggctacaccaactacaacccctccctggagtccaggatctccgtgaccagggacacctccaagaaccagttcttcctgcagctgaactccgtgaccaccgaggacaccgccacctactactgcgccagggaggtgggcctgaggctgggctggttcgcctactggggccagggcaccctggtggccgtgtccgccgccaagaccaccgccccctccgtgtaccccctggcccccgtgtgcggcgacaccaccggctcctccgtgaccctgggctgcctggtgaagggctacttccccgagcccgtgaccctgacctggaactccggctccctgtcctccggcgtgcacaccttccccgccgtgctgcagtccgacctgtacaccctgtcctcctccgtgaccgtgacctcctccacctggccctcccagtccatcacctgcaacgtggcccaccccgcctcctccaccaaggtggacaagaagatcgagcccaggggccccaccatcaagccctgccccccctgcaagtgccccgcccccaacctgctgggcggcccctccgtgttcatcttcccccccaagatcaaggacgtgctgatgatctccctgtcccccatcgtgacctgcgtggtggtggacgtgtccgaggacgaccccgacgtgcagatctcctggttcgtgaacaacgtggaggtgcacaccgcccagacccagacccacagggaggactacaactccaccctgagggtggtgtccgccctgcccatccagcaccaggactggatgtccggcaaggagttcaagtgcaaggtgaacaacaaggacctgcccgcccccatcgagaggaccatctccaagcccaagggctccgtgagggccccccaggtgtacgtgctgcccccccccgaggaggagatgaccaagaagcaggtgaccctgacctgcatggtgaccgacttcatgcccgaggacatctacgtggagtggaccaacaacggcaagaccgagctgaactacaagaacaccgagcccgtgctggactccgacggctcctacttcatgtactccaagctgagggtggagaagaagaactgggtggagaggaactcctactcctgctccgtggtgcacgagggcctgcacaaccaccacaccaccaagtccttctccaggacccccggcaag

SEQ ID NO: 51 - DNA, 642 bp, synthetic construct
  source 1..642: mol_type = other DNA
tccatcgtgatgacccagacccccaagttcctgctgatctccgccggcgacagggtgaccatcacctgcaaggcctcccagtccgtgaacaacgacgtggcctggtaccagcagaagcccggccagtcccccaagctgctgatctactacgcctccaacaggtacaccggcgtgcccgaccacttcaccggctccggctacggcaccgacttcaccttcaccatctccaccgtgcaggccgaggacctggccgtgtacttctgccagcagcactactcctccccctggaccttcggcggcggcaccaagctggagttcaagagggccgacgccgcccccaccgtgtccatcttccccccctcctccgagcagctgacctccggcggcgcctccgtggtgtgcttcctgaacaacttctaccccaaggacatcaacgtgaagtggaagatcgacggctccgagaggcagaacggcgtgctgaactcctggaccgaccaggactccaaggactccacctactccatgtcctccaccctgaccctgaccaaggacgagtacgagaggcacaactcctacacctgcgaggccacccacaagacctccacctcccccatcgtgaagtccttcaacaggaacgagtgc

SEQ ID NO: 52 - DNA, 1350 bp, synthetic construct
  source 1..1350: mol_type = other DNA
gacgtgcagctgcaggagtccggccccggcctggtgaagccctcccagtccctgtccctgacctgcaccgtgaccggctactccatcacctccgactacgcctggaactggatcaggcagttccccggcaacaagctggagtggatgggctacatctcctactccggctacaccaactacaacccctccctggagtccaggatctccgtgaccagggacacctccaagaaccagttcttcctgcagctgaactccgtgaccaccgaggacaccgccacctactactgcgccagggaggtgggcctgaggctgggctggttcgcctactggggccagggcaccctggtggccgtgtccgccgcctccaccaagggcccctccgtgttccccctggccccctcctccaagtccacctccggcggcaccgccgccctgggctgcctggtgaaggactacttccccgagcccgtgaccgtgtcctggaactccggcgccctgacctccggcgtgcacaccttccccgccgtgctgcagtcctccggcctgtactccctgtcctccgtggtgaccgtgccctcctcctccctgggcacccagacctacatctgcaacgtgaaccacaagccctccaacaccaaggtggacaagaaggtggagcccaagtcctgcgacaagacccacacctgccccccctgccccgcccccgagctgctgggcggcccctccgtgttcctgttcccccccaagcccaaggacaccctgatgatctccaggacccccgaggtgacctgcgtggtggtggacgtgtcccacgaggaccccgaggtgaagttcaactggtacgtggacggcgtggaggtgcacaacgccaagaccaagcccagggaggagcagtacaactccacctacagggtggtgtccgtgctgaccgtgctgcaccaggactggctgaacggcaaggagtacaagtgcaaggtgtccaacaaggccctgcccgcccccatcgagaagaccatctccaaggccaagggccagcccagggagccccaggtgtacaccctgcccccctccagggacgagctgaccaagaaccaggtgtccctgacctgcctggtgaagggcttctacccctccgacatcgccgtggagtgggagtccaacggccagcccgagaacaactacaagaccaccccccccgtgctggactccgacggctccttcttcctgtactccaagctgaccgtggacaagtccaggtggcagcagggcaacgtgttctcctgctccgtgatgcacgaggccctgcacaaccactacacccagaagtccctgtccctgtcccccggcaag

SEQ ID NO: 53 - DNA, 642 bp, synthetic construct
  source 1..642: mol_type = other DNA
tccatcgtgatgacccagacccccaagttcctgctgatctccgccggcgacagggtgaccatcacctgcaaggcctcccagtccgtgaacaacgacgtggcctggtaccagcagaagcccggccagtcccccaagctgctgatctactacgcctccaacaggtacaccggcgtgcccgaccacttcaccggctccggctacggcaccgacttcaccttcaccatctccaccgtgcaggccgaggacctggccgtgtacttctgccagcagcactactcctccccctggaccttcggcggcggcaccaagctggagttcaagaggaccgtggccgccccctccgtgttcatcttccccccctccgacgagcagctgaagtccggcaccgcctccgtggtgtgcctgctgaacaacttctaccccagggaggccaaggtgcagtggaaggtggacaacgccctgcagtccggcaactcccaggagtccgtgaccgagcaggactccaaggactccacctactccctgtcctccaccctgaccctgtccaaggccgactacgagaagcacaaggtgtacgcctgcgaggtgacccaccagggcctgtcctcccccgtgaccaagtccttcaacaggggcgagtgc

SEQ ID NO: 54 - DNA, 1437 bp, synthetic construct
  source 1..1437: mol_type = other DNA
gacatccagatgacccagtccccctcctccctgtccgcctccgtgggcgacagggtgaccatcacctgcaaggcctcccagtccgtgaacaacgacgtggcctggtaccagcagaagcccggcaaggcccccaagctgctgatctactacgcctccaacaggtacaccggcgtgccctccaggttctccggctccggctccggcaccgacttcaccttcaccatctcctccctgcagcccgaggacatcgccacctactactgccagcagcactactcctccccctggaccttcggctgcggcaccaagctggagatcaagggcggcggcggctccggcggcggcggctccggcggcggcggctccggcggcggcggctcccaggtgcagctgcaggagtccggccccggcctggtgaagccctccgagaccctgtccctgacctgcaccgtgtccggctactccatcacctccgactacgcctggaactggatcaggcagccccccggcaagtgcctggagtggatgggctacatctcctactccggctacaccaactacaacccctccctggagtccagggtgaccatctccagggacacctccaagaaccagttctccctgaagctgtcctccgtgaccgccgccgacaccgccgtgtactactgcgccagggaggtgggcctgaggctgggctggttcgcctactggggccagggcaccctggtgaccgtgtcctccgagcccaagtcctgcgacaagacccacacctgccccccctgccccgcccccgaggccgccggcggcccctccgtgttcctgttcccccccaagcccaaggacaccctgatgatctccaggacccccgaggtgacctgcgtggtggtggacgtgtcccacgaggaccccgaggtgaagttcaactggtacgtggacggcgtggaggtgcacaacgccaagaccaagcccagggaggagcagtacaactccacctacagggtggtgtccgtgctgaccgtgctgcaccaggactggctgaacggcaaggagtacaagtgcaaggtgtccaacaaggccctgcccgcccccatcgagaagaccatctccaaggccaagggccagcccagggagccccaggtgtacaccctgcccccctgcagggaggagatgaccaagaaccaggtgtccctgtggtgcctggtgaagggcttctacccctccgacatcgccgtggagtgggagtccaacggccagcccgagaacaactacaagaccaccccccccgtgctggactccgacggctccttcttcctgtactccaagctgaccgtggacaagtccaggtggcagcagggcaacgtgttctcctgctccgtgatgcacgaggccctgcacaaccactacacccagaagtccctgtccctgtcccccggcaag

SEQ ID NO: 55 - DNA, 1428 bp, synthetic construct
  source 1..1428: mol_type = other DNA
gacatccagatgacccagtccccctcctccctgtccgcctccgtgggcgacagggtgaccatcacctgctccgcctcccaggacatctccaactacctgaactggtaccagcagaagcccggcaaggcccccaagctgctgatctactacacctccaacctgcactccggcgtgccctccaggttctccggctccggctccggcaccgacttcaccctgaccatctcctccctgcagcccgaggacttcgccacctactactgccagcagtacaggaagctgccctggaccttcggccagggcaccaagctggagatcaagaggggcggcggcggctccggcggcggcggctccggcggcggcggctcccaggtgcagctggtgcagtccggcgccgaggtgaagaagcccggctcctccgtgaaggtgtcctgcaaggcctccggcggcaccttctccaactactggatgcactgggtgaggcaggcccccggccagggcctggagtggatgggcgccacctacaggggccactccgacacctactacaaccagaagttcaagggcagggtgaccatcaccgccgacaagtccacctccaccgcctacatggagctgtcctccctgaggtccgaggacaccgccgtgtactactgcgccaggggcgccatctacgacggctacgacgtgctggacaactggggccagggcaccctggtgaccgtgtcctccgagcccaagtcctgcgacaagacccacacctgccccccctgccccgcccccgaggccgccggcggcccctccgtgttcctgttcccccccaagcccaaggacaccctgatgatctccaggacccccgaggtgacctgcgtggtggtggacgtgtcccacgaggaccccgaggtgaagttcaactggtacgtggacggcgtggaggtgcacaacgccaagaccaagcccagggaggagcagtacaactccacctacagggtggtgtccgtgctgaccgtgctgcaccaggactggctgaacggcaaggagtacaagtgcaaggtgtccaacaaggccctgcccgcccccatcgagaagaccatctccaaggccaagggccagcccagggagccccaggtgtgcaccctgcccccctccagggaggagatgaccaagaaccaggtgtccctgtcctgcgccgtgaagggcttctacccctccgacatcgccgtggagtgggagtccaacggccagcccgagaacaactacaagaccaccccccccgtgctggactccgacggctccttcttcctggtgtccaagctgaccgtggacaagtccaggtggcagcagggcaacgtgttctcctgctccgtgatgcacgaggccctgcacaaccactacacccagaagtccctgtccctgtcccccggcaag

SEQ ID NO: 56 - DNA, 1434 bp, synthetic construct
  source 1..1434: mol_type = other DNA
gacatcgtgctgacccagacccccctgtccctgtccgtgacccccggccagcccgcctccatctcctgcaaggcctcccagtccgtggactacgacggcgactcctacatgaactggtacctgcagaagcccggccagcccccccagctgctgatctacgccgcctccaccctgcactccggcatccccgacaggttctccggctccggctccggcaccgacttcaccctgaagatctccagggtggaggccgaggacgtgggcgtgtactactgccagcagtccaaggaggaccccaggaccttcggccagggcaccaagctggagatcaagggcggcggcggctccggcggcggcggctccggcggcggcggctccgaggtgcagctggtgcagtccggcgccgaggtgaagaagcccggcgcctccgtgaaggtgtcctgcaaggcctccggctacaccttcaccgactacaacatggactgggtgaggcaggcccccggccagggcctggagtggatcggcgacatcaaccccaacaacggcggcaccctgtacaaccagaagttcaggggcagggtgaccctgaccgtggacacctccatctccaccgcctacatggagctgtccaggctgaggtccgacgacaccgccgtgtactactgcgccaggtccgaggtgttctacggcaactacgccgactactggggccagggcaccaccgtgaccgtgtcctccgagcccaagtcctgcgacaagacccacacctgccccccctgccccgcccccgaggccgccggcggcccctccgtgttcctgttcccccccaagcccaaggacaccctgatgatctccaggacccccgaggtgacctgcgtggtggtggacgtgtcccacgaggaccccgaggtgaagttcaactggtacgtggacggcgtggaggtgcacaacgccaagaccaagcccagggaggagcagtacaactccacctacagggtggtgtccgtgctgaccgtgctgcaccaggactggctgaacggcaaggagtacaagtgcaaggtgtccaacaaggccctgcccgcccccatcgagaagaccatctccaaggccaagggccagcccagggagccccaggtgtgcaccctgcccccctccagggaggagatgaccaagaaccaggtgtccctgtcctgcgccgtgaagggcttctacccctccgacatcgccgtggagtgggagtccaacggccagcccgagaacaactacaagaccaccccccccgtgctggactccgacggctccttcttcctggtgtccaagctgaccgtggacaagtccaggtggcagcagggcaacgtgttctcctgctccgtgatgcacgaggccctgcacaaccactacacccagaagtccctgtccctgtcccccggcaag

SEQ ID NO: 57 - DNA, 870 bp, synthetic construct
  source 1..870: mol_type = other DNA
atgggtggaggggctggggaaaggctgtttacttcctcctgtctagtcggtttggtccctttagggctccggatatctttggtgacttgtccactccagtgtggcatcatgtggcagctgctcctcccaactgctctgctacttctagtttcagctggcatgcggactgaagatctcccaaaggctgtggtgttcctggagcctcaatggtacagggtgctcgagaaggacagtgtgactctgaagtgccagggagcctactcccctgaggacaattccacacagtggtttcacaatgagagcctcatctcaagccaggcctcgagctacttcattgacgctgccacagtcgacgacagtggagagtacaggtgccagacaaacctctccaccctcagtgacccggtgcagctagaagtccatatcggctggctgttgctccaggcccctcggtgggtgttcaaggaggaagaccctattcacctgaggtgtcacagctggaagaacactgctctgcataaggtcacatatttacagaatggcaaaggcaggaagtattttcatcataattctgacttctacattccaaaagccacactcaaagacagcggctcctacttctgcagggggctttttgggagtaaaaatgtgtcttcagagactgtgaacatcaccatcactcaaggtttggcagtgtcaaccatctcatcattctttccacctgggtaccaagtctctttctgcttggtgatggtactcctttttgcagtggacacaggactatatttctctgtgaagacaaacattcgaagctcaacaagagactggaaggaccataaatttaaatggagaaaggaccctcaagacaaa

SEQ ID NO: 58 - DNA, 765 bp, synthetic construct
  source 1..765: mol_type = other DNA
atgtggcagctgctcctcccaactgctctgctacttctagtttcagctggcatgcgggctgaagatctcccaaaggctgtggtgttcctggagcctcaatggtacagggtgctcgagaaggaccgtgtgactctgaagtgccagggagcctactcccctgaggacaattccacacggtggtttcacaatgagagcctcatctcaagccagacctcgagctacttcattgctgctgccagagtcaacaacagtggagagtacaggtgccagacaagcctctccacactcagtgacccggtgcagctggaagtccatatcggctggctattgctccaggcccctcggtgggtgttcaaggaggaagaatctattcacctgaggtgtcacagctggaagaacactcttctgcataaggtcacgtatttacagaatggcaaaggcaggaagtattttcatcagaattctgacttctacattccaaaagccacactcaaagacagcggctcctacttctgcaggggacttattgggagtaaaaatgtatcttcagagactgtgaacatcaccatcactcaagatttggcagtgtcatccatctcatcattctttccacctgggtaccaagtctctttctgcctggtgatggtactcctttttgcagtggacacaggactatatttctctatgaagaaaagcattccaagctcaacaagggactgggaggaccataaatttaaatggagcaaggaccctcaagacaaatga

SEQ ID NO: 59 - protein, 121 aa, synthetic construct
QVQLVQSGAEVKKPGSSVKVSCKASGGTFSNYWMHWVRQAPGQGLEWMGATYRGHSDTYYNQKFKGRVTITADKSTSTAYMELSSLRSEDTAVYYCARGAIYDGYDVLDNWGQGTLVTVSS

SEQ ID NO: 60 - protein, 111 aa, synthetic construct
DIVLTQTPLSLSVTPGQPASISCKASQSVDYDGDSYMNWYLQKPGQPPQLLIYAASTLHSGIPDRFSGSGSGTDFTLKISRVEAEDVGVYYCQQSKEDPRTFGQGTKLEIK

SEQ ID NO: 61 - protein, 120 aa, synthetic construct
EVQLVQSGAEVKKPGASVKVSCKASGYTFTDYNMDWVRQAPGQGLEWIGDINPNNGGTLYNQKFRGRVTLTVDTSISTAYMELSRLRSDDTAVYYCARSEVFYGNYADYWGQGTTVTVSS

SEQ ID NO: 62 - protein, 111 aa, synthetic construct; identical to SEQ ID NO: 60